European Patent Application EP 4 424 319 A2, published September 4, 2024. Title: Novel lactic acid bacteria with various functionality and use thereof. Applicant: Navipharm Co, Ltd. Application EP. The sequence listing filed with the application follows.

SEQUENCE LISTING (12 sequences)

SEQ ID NO: 1 - DNA, 1132 bp, synthetic construct
  misc_feature 1..1132: note = 16S rDNA of Lactobacillus brevis CH23
  source 1..1132: mol_type = other DNA
agggataacacttggaaacaggtgctaataccgtataacaacaaaatccgcatggattttgtttgaaaggtggcttcggctatcacttctggatgatcccgcggcgtattagttagttggtgaggtaaaggcccaccaagacgatgatacgtagccgacctgagagggtaatcggccacattgggactgagacacggcccaaactcctacgggaggcagcagtagggaatcttccacaatggacgaaagtctgatggagcaatgccgcgtgagtgaagaagggtttcggctcgtaaaactctgttgttaaagaagaacacctttgagagtaactgttcaagggttgacggtatttaaccagaaagccacggctaactacgtgccagcagccgcggtaatacgtaggtggcaagcgttgtccggatttattgggcgtaaagcgagcgcaggcggttttttaagtctgatgtgaaagccttcggcttaaccggagaagtgcatcggaaactgggagacttgagtgcagaagaggacagtggaactccatgtgtagcggtggaatgcgtagatatatggaagaacaccagtggcgaaggcggctgtctagtctgtaactgacgctgaggctcgaaagcatgggtagcgaacaggattagataccctgstagtccatgccgtaaacgatgagtgctaagtgttggagggtttccgcccttcagtgctgcagctaacgcattaagcactccgcctggggagtacgaccgcaaggttgaaactcaaaggaattgacgggggcccgcacaagcggtggagcatgtggtttaattcgaagctacgcgaagaaccttaccaggtcttgacatcttctgccaatcttagagataagacgttcccttcggggacagaatgacaggtggtgcatggttgtcgtcagctcgtgtcgtgagatgttgggttaagtcccgcaacgagcgcaacccttattatcagttgccagcattcagttgggcactctggtgagactgccggtgacaaaccggaggaaggtggggatgacgtcaaatcatcatgccccttatgacctgggctacacacgtgctacaatggacggtacaacgagtcgcgaagtcgt

SEQ ID NO: 2 - DNA, 1258 bp, synthetic construct
  misc_feature 1..1258: note = 16S rDNA of Lactobacillus johnsonii CH32
  source 1..1258: mol_type = other DNA
gtaacttgcccaagagactgggataacacctggaaacagatgctaataccggataacaacactagacgcatgtctagagtttgaaagatggttctgctatcactcttggatggacctgcggtgcattagctagttggtaaggtaacggcttaccaaggcaatgatgcatagccgagttgagagactgatcggccacattgggactgagacacggcccaaactcctacgggaggcagcagtagggaatcttccacaatggacgaaagtctgatggagcaacgccgcgtgagtgaagaagggtttcggctcgtaaagctctgttggtagtgaagaaagatagaggtagtaactggccttgatttgacggtaattccccagaaagtcacggctaactacgtgccagcagccgcggtaatacgtaggtggcaagcgttgtccggatttattgggcgtaaagcgagtgcaggcggttcaataagtctgatgtgaaagccttcggctcaaccggagaattgcatcagaaactgttgaacttgagtgcagaagaggagagtggaactccatgtgtagcggtggaatgcgtagatatatggaagaacaccagtggcgaaggcggctctctggtctgcaactgacgctgaggctcgaaagcatgggtagcgaacaggattagataccctggtagtccatgccgtaaacgatgagtgctaagtgttgggaggtttccgcctctcagtgctgcagctaacgcattaagcactccgcctggggagtacgaccgcaaggttgaaactcaaaggaattgacgggggcccgcacaagcggtggagcatgtggtttaattcgaagcaacgcgaagaaccttaccaggtcttgacatccagtgcaaacctaagagattaggtgttcccttcggggacgctgagacaggtggtgcatggctgtcgtcagctcgtgtcgtgagatgttgggttaagtcccgcaacgagcgcaacccttgtcattagttgccatcattaagttgggcactctaatgagactgccggtgacaaaccggaggaaggtggggatgacgtcaagtcatcatgccccttatgacctgggctacacacgtgctacaatggacggtacaacgagaagcgaacctgcgaaggcaagcggatctcttaaagccgttctcagttcggactgtaggctgcaactcgcctacacgaagctggaatcgctagtaatcgcggaacagtacgccgcggtgaat

SEQ ID NO: 3 - DNA, 1348 bp, synthetic construct
  misc_feature 1..1348: note = 16S rDNA of Bifidobacterium longum CH57
  source 1..1348: mol_type = other DNA
cgggctttgcttggtggtgagagtggcgaacgggtgagtaatgcgtgaccgacctgccccatacaccggaatagctcctggaaacgggtggtaatgccggatgctccagttgatcgcatggtcttctgggaaagctttcgcggtatgggatggggtcgcgtcctatcagcttgacggcggggtaacggcccaccgtggcttcgacgggtagccggcctgagagggcgaccggccacattgggactgagatacggcccagactcctacgggaggcagcagtggggaatattgcacaatgggcgcaagcctgatgcagcgacgccgcgtgagggatggaggccttcgggttgtaaacctcttttatcggggagcaagcgagagtgagtttacccgttgaataagcaccggctaactacgtgccagcagccgcggtaatacgtagggtgcaagcgttatccggaattattgggcgtaaagggctcgtaggcggttcgtcgcgtccggtgtgaaagtccatcgcttaacggtggatccgcgccgggtacgggcgggcttgagtgcggtaggggagactggaattcccggtgtaacggtggaatgtgtagatatcgggaagaacaccaatggcgaaggcaggtctctgggccgttactgacgctgaggagcgaaagcgtggggagcgaacaggattagataccctggtagtccacgccgtaaacggtggatgctggatgtggggcccgttccacgggttccgtgtcggagctaacgcgttaagcatcccgcctgggggagtacggccgcaaggctaaaactcaaagaaattgacgggggcccgcacaagcggcggagcatgcggattaattcgatgcaacgcgaagaaccttacctgggcttcacatgttcccgacggtcgtagagatacggcttcccttcggggcgggttcacaggtggtgcatggtcgtcgtcagctcgtgtcgtgagatgttgggttaagtcccgcaacgagcgcaaccctcgccccgtgttgccagcggattatgccgggaactcacgggggaccgccggggttaactcggaggaaggtggggatgacgtcagatcatcatgccccttacgtccagggcttcacgcatgctacaatggccggtacaacgggatgcgacgcggcgacgcggagcggatccctgaaaaccggtctcagttcggatcgcagtctgcaactcgactgcgtgaaggcggagtcgctagtaatcgcgaatcagcaacgtcgcggtgaatgcgttcccgggccttgtacacaccgcccgtcaagtcatgaaagtgggcagcacccgaagccggtgg

SEQ ID NO: 4 - DNA, 1421 bp, synthetic construct
  misc_feature 1..1421: note = 16S rDNA of Lactobacillus plantarum LC5
  source 1..1421: mol_type = other DNA
ctggtattgattggtgcttgcatcatgatttacatttgagtgagtggcgaactggtgagtaacacgtgggaaacctgcccagaagcgggggataacacctggaaacagatgctaataccgcataacaacttggaccgcatggtccgagcttgaaagatggcttcggctatcacttttggatggtcccgcggcgtattagctagatggtggggtaacggctcaccatggcaatgatacgtagccgacctgagagggtaatcggccacattgggactgagacacggcccaaactcctacgggaggcagcagtagggaatcttccacaatggacgaaagtctgatggagcaacgccgcgtgagtgaagaagggtttcggctcgtaaaactctgttgttaaagaagaacatatctgagagtaactgttcaggtattgacggtatttaaccagaaagccacggctaactacgtgccagcagccgcggtaatacgtaggtggcaagcgttgtccgggatttattgggcgtaaagcgagcgcaggcggttttttaagtctgatgtgaaagccttcggctcaaccgaagaagtgcatcggaaactgggaaacttgagtgcagaagaggacagtggaactccatgtgtagcggtgaaatgcgtagatatatggaagaacaccagtggcgaaggcggctgtctggtctgtaactgacgctgaggctcgaaagtatgggtagcaaacaggattagataccctggtagtccataccgtaaacgatgaatgctaagtgttggagggtttccgcccttcagtgctgcagctaacgcattaagcattccgcctggggagtacggccgcaaggctgaaactcaaaggaattgacgggggcccgcacaagcggtggagcatgtggtttaattcgaagctacgcgaagaaccttaccaggtcttgacatactatgcaaatctaagagattagacgttcccttcggggacatggatacaggtggtgcatggttgtcgtcagctcgtgtcgtgagatgttgggttaagtcccgcaacgagcgcaacccttattatcagttgccagcattaagttgggcactctggtgagactgccggtgacaaaccggaggaaggtggggatgacgtcaaatcatcatgccccttatgacctgggctacacacgtgctacaatggatggtacaacgagttgcgaactcgcgagagtaagctaatctcttaaagccattctcagttcggattgtaggctgcaactcgcctacatgaagtcggaatcgctagtaatcgcggatcagcatgccgcggtgaatacgttcccgggccttgtacacaccgcccgtcacaccatgagagtttgtaacacccaaagtcggtggggtaaccttttaggaaccagccgcct

SEQ ID NO: 5 - DNA, 1356 bp, synthetic construct
  misc_feature 1..1356: note = 16S rDNA of Lactobacillus plantarum LC27
  source 1..1356: mol_type = other DNA
tttacatttgattgagtggcgaactggtgagtaacacgtgggaaacctgcccagaagcgggggataacacctggaaacagatgctaataccgcataacaacttggaccgcatggtccgagtttgaaagatggcttcggctatcacttttggatggtcccgcggcgtattagctagatggtggggtaacggctcaccatggcaatgatacgtagccgacctgagagggtaatcggccacattgggactgagacacggcccaaactcctacgggaggcagcagtagggaatcttccacaatggacgaaagtctgatggagcaacgccgcgtgagtgaagaagggtttcggctcgtaaaactctgttgttaaagaagaacatatctgagagtaactgttcaggtattgacggtatttaaccagaaagccacggctaactacgtgccagcagccgcggtaatacgtaggtggcaagcgttgtccggatttattgggcgtaaagcgagcgcaggcggttttttaagtctgatgtgaaagccttcggctcaaccgaagaagtgcatcggaaactgggaaacttgagtgcagaagaggacagtggaactccatgtgtagcggtgaaatgcgtagatatatggaagaacaccagtggcgaaggcggctgtctggtctgtaactgacgctgaggctcgaaagtatgggtagcaaacaggattagataccctggtagtccataccgtaaacgatgaatgctaagtgttggagggtttccgcccttcagtgctgcagctaacgcattaagcattccgcctggggagtacggccgcaaggctgaaactcaaaggaattgacgggggcccgcacaagcggtggagcatgtggtttaattcgaagctacgcgaagaaccttaccaggtcttgacatactatgcaaatctaagagattagacgttcccttcggggacatggatacaggtggtgcatggttgtcgtcagctcgtgtcgtgagatgttgggttaagtcccgcaacgagcgcaacccttattatcagttgccagcattaagttgggcactctggtgagactgccggtgacaaaccggaggaaggtggggatgacgtcaaatcatcatgccccttatgacctgggctacacacgtgctacaatggatggtacaacgagttgcgaactcgcgagagtaagctaatctcttaaagccattctcagttcggattgtaggctgcaactcgcctacatgaagtcggaatcgctagtaatcgcggatcagcatgccgcggtgaatacgttcccgggccttgtacacaccgcccgtcacaccatgagagtttgtaacaccca

SEQ ID NO: 6 - DNA, 1325 bp, synthetic construct
  misc_feature 1..1325: note = 16S rDNA of Lactobacillus plantarum LC28
  source 1..1325: mol_type = other DNA
catcatgatttacatttgagtgagtggcgaactggtgagtaacacgtgggaaacctgcccagaagcgggggataacacctggaaacagatgctaataccgcataacaacttggaccgcatggtccgagtttgaaagatggcttcggctatcacttttggatggtcccgcggcgtattagctagatggtggggtaacggctcaccatggcaatgatacgtagccgacctgagagggtaatcggccacattgggactgagacacggcccaaactcctacgggaggcagcagtagggaatcttccacaatggacgaaagtctgatggagcaacgccgcgtgagtgaagaagggtttcggctcgtaaaactctgttgttaaagaagaacatatctgagagtaactgttcaggtattgacggtatttaaccagaaagccacggctaactacgtgccagcagccgcggtaatacgtaggtggcaagcgttgtccggatttattgggcgtaaagcgagcgcaggcggttttttaagtctgatgtgaaagccttcggctcaaccgaagaagtgcatcggaaactgggaaacttgagtgcagaagaggacagtggaactccatgtgtagcggtgaaatgcgtagatatatggaagaacaccagtggcgaaggcggctgtctggtctgtaactgacgctgaggctcgaaagtatgggtagcaaacaggattagataccctggtagtccataccgtaaacgatgaatgctaagtgttggagggtttccgcccttcagtgctgcagctaacgcattaagcattccgcctggggagtacggccgcaaggctgaaactcaaaggaattgacgggggcccgcacaagcggtggagcatgtggtttaattcgaagctacgcgaagaaccttaccaggtcttgacatactatgcaaatctaagagattagacgttcccttcggggacatggatacaggtggtgcatggttgtcgtcagctcgtgtcgtgagatgttgggttaagtcccgcaacgagcgcaacccttattatcagttgccagcattaagttgggcactctggtgagactgccggtgacaaaccggaggaaggtggggatgacgtcaaatcatcatgccccttatgacctgggctacacacgtgctacaatggatggtacaacgagttgcgaactcgcgagagtaagctaatctcttaaagccattctcagttcggattgtaggctgcaactcgcctacatgaagtcggaatcgctagtaatcgcggatcagcattccgcggtgaatacgttcccgggccttgt

SEQ ID NO: 7 - DNA, 1342 bp, synthetic construct
  misc_feature 1..1342: note = 16S rDNA of Bifidobacterium longum LC67
  source 1..1342: mol_type = other DNA
ggctttgcttggtggtgagagtggcgaacgggtgagtaatgcgtgaccgacctgccccatacaccggaatagctcctggaaacgggtggtaatgccggatgctccagttgatcgcatggtcttctgggaaagctttcgcggtatgggatggggtcgcgtcctatcagcttgacggcggggtaacggcccaccgtggcttcgacgggtagccggcctgagagggcgaccggccacattgggactgagatacggcccagactcctacgggaggcagcagtggggaatattgcacaatgggcgcaagcctgatgcagcgacgccgcgtgagggatggaggccttcgggttgtaaacctcttttatcggggagcaagcgagagtgagtttacccgttgaataagcaccggctaactacgtgccagcagccgcggtaatacgtagggtgcaagcgttatcccggaattattgggcgtaaagggctcgtaggcggttcgtcgcgtccggtgtgaaagtccatcgcttaacggtggatccgcgccgggtacgggcgggcttgagtgcggtaggggagactggaattcccggtgtaacggtggaatgtgtagatatcgggaagaacaccaatggcgaaggcaggtctctgggccgttactgacgctgaggagcgaaagcgtggggagcgaacaggattagataccctggtagtccacgccgtaaacggtggatgctggatgtggggcccgttccacgggttccgtgtcggagctaacgcgttaagcatcccgcctgggggagtacggccgcaaggctaaaactcaaagaaattgacgggggcccgcacaagcggcggagcatgcggattaattcgatgcaacgcgaagaaccttacctgggcttgacatgttcccgacggtcgtagagatacggcttcccttcggggcgggttcacaggtggtgcatggtcgtcgtcagctcgtgtcgtgagatgttgggttaagtcccgcaacgagcgcaaccctcgccccgtgttgccagcggattatgccgggaactcacgggggaccgccggggttaactcggaggaaggtggggatgacgtcagatcatcatgccccttacgtccagggcttcacgcatgctacaatggccggtacaacgggatgcgacgcggcgacgcggagcggatccctgaaaaccggtctcagttcggatcgcagtctgcaactcgactgcgtgaaggcggagtcgctagtaatcgcgaatcagcaacgtcgcggtgaatgcgttcccgggccttgtacacaccgcccgtcaagtcatgaaagtgggcagcacccgaagcg

SEQ ID NO: 8 - DNA, 1343 bp, synthetic construct
  misc_feature 1..1343: note = 16S rDNA of Bifidobacterium longum LC68
  source 1..1343: mol_type = other DNA
cggcttcgggtgctgcccactttcatgacttgacgggcggtgtgtacaaggcccgggaacgcattcaccgcgacgttgctgattcgcgattactagcgactccgccttcacgcagtcgagttgcagactgcgatccgaactgagaccggttttcagggatccgctccgcgtcgccgcgtcgcatcccgttgtaccggccattgtagcatgcgtgaagccctggacgtaaggggcatgatgatctgacgtcatccccaccttcctccgagttaaccccggcggtcccccgtgagttcccggcataatccgctggcaacacggggcgagggttgcgctcgttgcgggacttaacccaacatctcacgacacgagctgacgacgaccatgcaccacctgtgaacccgccccgaagggaagccgcatctctacgaccgtcgggaacatgtcaagcccaggtaaggttcttcgcgttgcatcgaattaatccgcatgctccgccgcttgtgcgggcccccgtcaatttctttgagttttagccttgcggccgtactccccaggcgggatgcttaacgcgttagctccgacacggaacccgtggaacgggccccacatccagcatccaccgtttacggcgtggactaccagggtatctaatcctgttcgctccccacgctttcgctcctcagcgtcagtaacggcccagagacctgccttcgccattggtgttcttcccgatatctacacattccaccgttacaccgggaattccagtctcccctaccgcactcaagcccgcccgtacccggcgcggatccaccgttaagcgatggactttcacaccggacgcgacgaaccgcctacgagccctttacgcccaataattccggataacgcttgcaccctacgtattaccgcggctgctggcacgtagttagccggtgcttattcaacgggtaaactcactctcgcttgctccccgataaaagaggtttacaacccgaaggcctccatccctcacgcggcgtcgctgcatcaggcttgcgcccattgtgcaatattccccactgctgcctcccgtaggagtctgggccgtatctcagtcccaatgtggccggtcgccctctcaggccggctacccgtcgaagccacggtgggccgttaccccgccgtcaagctgataggacgcgaccccatcccataccgcgaaagctttcccagaagaccatgcgatcaactggagcatccggcattaccacccgtttccaggagctattccggtgtatggggcaggtcggtcacgcattactcacccgttcgccactctcaccaccaagcaaagtctc

SEQ ID NO: 9 - DNA, 19 bp, synthetic construct
  misc_feature 1..19: note = TNF-alpha forward primer
  source 1..19: mol_type = other DNA
ctgtagcccacgtcgtagc

SEQ ID NO: 10 - DNA, 18 bp, synthetic construct
  misc_feature 1..18: note = TNF-alpha reverse primer
  source 1..18: mol_type = other DNA
ttgagatccatgccgttg

SEQ ID NO: 11 - DNA, 20 bp, synthetic construct
  misc_feature 1..20: note = CXCL4 forward primer
  source 1..20: mol_type = other DNA
agtcctgagctgctgcttct

SEQ ID NO: 12 - DNA, 20 bp, synthetic construct
  misc_feature 1..20: note = CXCL4 reverse primer
  source 1..20: mol_type = other DNA
gatctccatcgctttcttcg